European Patent Application EP 4 379 062 A1, published June 5, 2024. Title: Biosystem for pesticide detection. Applicant: Fundacion AZTI – AZTI Fundazioa. The sequence listing filed with the application follows.

SEQUENCE LISTING (2 sequences)

SEQ ID NO: 1 - protein, 494 aa, Canis lupus
MELSVLLLLALLTGLLLLMARGHPKAYGHLPPGPRPLPILGNFLQMDRKGLLKSFLRLQEKYGDVFTVYLGPRRTVMLCGIDAIREALVDNAEAFSGRGKIAVVEPVFQGYGVVFANGERWKTLRRFSLATMRDFGMGKRSVEERIQEEAQCLVEELRKTEGVLQDPTFFFHSMTANIICSIVFGKRFGYKDPEFLRLMNLFYVSFALISSFSSQMFELFHSFLKYFPGTHRQVYNNLQEIKAFIARMVEKHRETLDPSAPRDFIDAYLIRMDKEKAEPSSEFHHRNLIDTALSLFFAGTETTSTTLRYGFLLMLKYPHIAERIYKEIDQVIGPHRLPSLDDRAKMPYTDAVIHEIQRFGDLLPIGVPHMVTKDICFRGYIIPKGTEVFPILHSALNDPHYFEKPDVFNPDHFLDANGALKKNEAFIPFSIGKRICLGEGIARMELFLFFTTILQNFSVASPMAPEDIDLTPQEIGVGKLPPVYQISFLSRGGC

SEQ ID NO: 2 - protein, 491 aa, Mus musculus
MEPSVLLLLALLVGFLLLLARGHPKSRGNFPPGPRPLPLLGNLLQMDRGGLLKSFIQLREKYGDVFTVHLGPRPVVMLCGTDTIREALVGQAEAFSGRGTVAVVEPTFKEYGVIFANGERWKTLRRFSLATMRDFGMGKRSVEERIQEEAQCLVEELRKSQGAPLDPTFLFQCITANIICSIVFGERFEYTDRQFLRLLELFYQTFSLISSFSSQMFELFSGFLKYFPGAHRQISKNLQELLDYIGHSVEKHRATLDPSVPRDFIDIYLLRMEKEKSNQHTEFHHQNLMMSVLSLFFAGTETSSTTLRYGFLLMLKYPHVAEKVQKEIDQVIGSHRLPTLDDRTKMPYTDAVIHEIQRFSDLIPIGVPHRVTKDTMFRGYLLPKNTEVYPILSSALHDPQYFEQPDSFNPDHFLDANGALKKSEAFLPFSTGKRICLGESIARNELFLFFTSILQNFSVASHVAPKDIDLTPKESGIGKIPPTYQICFLAR